European Patent Application EP 4 269 611 A2, published November 1, 2023. Title: POLYNUCLEOTIDE ENRICHMENT AND AMPLIFICATION USING ARGONAUTE SYSTEMS. Applicant: ILLUMINA, INC. Application EP, filed July 31, 2023. The sequence listing filed with the application follows.

SEQUENCE LISTING (16 sequences)

SEQ ID NO: 1 - DNA, 29 bp, synthetic construct
  misc_feature 1..29: note = Standard P5 sequence
  source 1..29: mol_type = other DNA
aatgatacggcgaccaccgagatctacac

SEQ ID NO: 2 - DNA, 24 bp, synthetic construct
  misc_feature 1..24: note = Standard P7 sequence
  source 1..24: mol_type = other DNA
caagcagaagacggcatacgagat

SEQ ID NO: 3 - DNA, 32 bp, synthetic construct
  misc_feature 1..32: note = PAM-Modified P5 sequence
  misc_feature 3: note = n is a, c, g, or t
  source 1..32: mol_type = other DNA
ccnaatgatacggcgaccaccgagatctacac

SEQ ID NO: 4 - DNA, 27 bp, synthetic construct
  misc_feature 1..27: note = PAM-Modified P7 sequence
  misc_feature 3: note = n is a, c, g, or t
  source 1..27: mol_type = other DNA
ccncaagcagaagacggcatacgagat

SEQ ID NO: 5 - DNA, 21 bp, synthetic construct
  misc_feature 1..21: note = Truncated PAM-Modified P5 sequence
  misc_feature 3: note = n is a, c, g, or t
  source 1..21: mol_type = other DNA
ccnaatgatacggcgaccacc

SEQ ID NO: 6 - DNA, 21 bp, synthetic construct
  misc_feature 1..21: note = Truncated PAM-Modified P7 sequence
  misc_feature 3: note = n is a, c, g, or t
  source 1..21: mol_type = other DNA
ccncaagcagaagacggcata

SEQ ID NO: 7 - RNA, 20 nt, synthetic construct
  misc_feature 1..20: note = Guide RNA P5 targeting
  source 1..20: mol_type = other RNA
tcggtggtcgccgtatcatt

SEQ ID NO: 8 - RNA, 20 nt, synthetic construct
  misc_feature 1..20: note = Guide RNA P7 targeting
  source 1..20: mol_type = other RNA
cgtatgccgtcttctgcttg

SEQ ID NO: 9 - DNA, 27 bp, synthetic construct
  misc_feature 1..27: note = Nextra Amplicon in solution - Example anti-sense strand
  source 1..27: mol_type = other DNA
cctcaagcagaagacggcatacgagat

SEQ ID NO: 10 - DNA, 32 bp, synthetic construct
  misc_feature 1..32: note = Nextra Amplicon in solution - Example anti-sense strand
  source 1..32: mol_type = other DNA
gtgtagatctcggtggtcgccgtatcattagg

SEQ ID NO: 11 - DNA, 32 bp, synthetic construct
  misc_feature 1..32: note = Nextra Amplicon in solution - Example sense strand
  source 1..32: mol_type = other DNA
cctaatgatacggcgaccaccgagatctacac

SEQ ID NO: 12 - DNA, 27 bp, synthetic construct
  misc_feature 1..27: note = Nextra Amplicon in solution - Example sense strand
  source 1..27: mol_type = other DNA
atctcgtatgccgtcttctgcttgagg

SEQ ID NO: 13 - DNA, 26 bp, synthetic construct
  misc_feature 1..26: note = Nextera amplicon in solution - Cas9-mediated linear amplification P5 primer
  misc_feature 1..5: note = n is a, c, g, or t
  source 1..26: mol_type = other DNA
nnnnncctaatgatacggcgaccacc

SEQ ID NO: 14 - DNA, 37 bp, synthetic construct
  misc_feature 1..37: note = Nextera amplicon in solution - Cas9-mediated linear amplification P5 extended sequence
  misc_feature 1..5: note = n is a, c, g, or t
  source 1..37: mol_type = other DNA
nnnnncctaatgatacggcgaccaccgagatctacac

SEQ ID NO: 15 - DNA, 26 bp, synthetic construct
  misc_feature 1..26: note = Nextera amplicon in solution - Cas9-mediated linear amplification P7 primer
  misc_feature 1..5: note = n is a, c, g, or t
  source 1..26: mol_type = other DNA
nnnnncctcaagcagaagacggcata

SEQ ID NO: 16 - DNA, 32 bp, synthetic construct
  misc_feature 1..32: note = Nextera amplicon in solution - Cas9-mediated linear amplification P7 extended sequence
  misc_feature 1..5: note = n is a, c, g, or t
  source 1..32: mol_type = other DNA
nnnnncctcaagcagaagacggcatacgagat